European Patent Application EP 4 538 295 A2, published April 16, 2025. Title: ANTIGEN BINDING MOLECULES AND METHODS OF USE THEREOF. Applicant: KITE PHARMA, INC. The sequence listing filed with the application follows.

SEQUENCE LISTING (82 sequences)

SEQ ID NO: 1 - protein, 245 aa, synthetic construct
  REGION 1..245: note = Description of Artificial Sequence: Synthetic polypeptide
DIQMTQTTSSLSASLGDRVTISCRASQDISKYLNWYQQKPDGTVKLLIYHTSRLHSGVPSRFSGSGSGTDYSLTISNLEQEDIATYFCQQGNTLPYTFGGGTKLEITGSTSGSGKPGSGEGSTKGEVKLQESGPGLVAPSQSLSVTCTVSGVSLPDYGVSWIRQPPRKGLEWLGVIWGSETTYYNSALKSRLTIIKDNSKSQVFLKMNSLQTDDTAIYYCAKHYYYGGSYAMDYWGQGTSVTVSS

SEQ ID NO: 2 - DNA, 396 bp, synthetic construct
  misc_feature 1..396: note = Description of Artificial Sequence: Synthetic polynucleotide
  source 1..396: mol_type = other DNA
atggagactgggctgcgctggcttctcctggtcgctgtgctcaaaggtgtccagtgtcaggagcagctggaggagtccgggggagacctggtcaagcctggaggaaccctgacagtcacctgcaaagcctctggattctccttcagtaacaatggaatttgctgggtccgccaggctccagggaaggggctggagtggatcggatgtctttatgttggtagtagtgataccacttactacgcgagctgggcgaaaggccgattcaccatctccaaaagctcgtcgaccacggtgactctacaaatgaccagtctgacagtcgcggacacggccacctatttctgtacgataaatctcggcttgtggggccccggcaccctggtcaccgtctcctca

SEQ ID NO: 3 - protein, 132 aa, synthetic construct
  REGION 1..132: note = Description of Artificial Sequence: Synthetic polypeptide
METGLRWLLLVAVLKGVQCQEQLEESGGDLVKPGGTLTVTCKASGFSFSNNGICWVRQAPGKGLEWIGCLYVGSSDTTYYASWAKGRFTISKSSSTTVTLQMTSLTVADTATYFCTINLGLWGPGTLVTVSS

SEQ ID NO: 4 - protein, 455 aa, synthetic construct
  REGION 1..455: note = Description of Artificial Sequence: Synthetic polypeptide
METGLRWLLLVAVLKGVQCQEQLEESGGDLVKPGGTLTVTCKASGFSFSNNGICWVRQAPGKGLEWIGCLYVGSSDTTYYASWAKGRFTISKSSSTTVTLQMTSLTVADTATYFCTINLGLWGPGTLVTVSSGQPKAPSVFPLAPCCGDTPSSTVTLGCLVKGYLPEPVTVTWNSGTLTNGVRTFPSVRQSSGLYSLSSVVSVTSSSQPVTCNVAHPATNTKVDKTVAPSTCSKPTCPPPELLGGPSVFIFPPKPKDTLMISRTPEVTCVVVDVSQDDPEVQFTWYINNEQVRTARPPLREQQFNSTIRVVSTLPIAHQDWLRGKEFKCKVHNKALPAPIEKTISKARGQPLEPKVYTMGPPREELSSRSVSLTCMINGFYPSDISVEWEKNGKAEDNYKTTPAVLDSDGSYFLYSKLSVPTSEWQRGDVFTCSVMHEALHNHYTQKSISRSPGK

SEQ ID NO: 5 - protein, 7 aa, synthetic construct
  REGION 1..7: note = Description of Artificial Sequence: Synthetic peptide
GFSFSNN

SEQ ID NO: 6 - protein, 6 aa, synthetic construct
  REGION 1..6: note = Description of Artificial Sequence: Synthetic peptide
YVGSSD

SEQ ID NO: 7 - protein, 4 aa, synthetic construct
  REGION 1..4: note = Description of Artificial Sequence: Synthetic peptide
NLGL

SEQ ID NO: 8 - DNA, 402 bp, synthetic construct
  misc_feature 1..402: note = Description of Artificial Sequence: Synthetic polynucleotide
  source 1..402: mol_type = other DNA
atggacacgagggcccccactcagctgctggggctcctgctgctctggctcccaggtgccacatttgccatcgtggtgacccagactccatcttccaagtctgtccctgtgggaggcacagtcaccatcaattgccaggccagtgagagtgtttataatagcgactggttagcctggtatcagcagaaaccagggcagcctcccaagcaactgatctatgctgcatccactctggcatctggggtcccatcgcgcttcaaaggcagtggatctgggacacagttcactctcaccatcagcgatgtggtgtgtgacgatgctgccacttattattgtgcaggatataaaagtagtagtactgatgggattgctttcggcggagggaccgaggtggtggtcaaa

SEQ ID NO: 9 - protein, 134 aa, synthetic construct
  REGION 1..134: note = Description of Artificial Sequence: Synthetic polypeptide
MDTRAPTQLLGLLLLWLPGATFAIVVTQTPSSKSVPVGGTVTINCQASESVYNSDWLAWYQQKPGQPPKQLIYAASTLASGVPSRFKGSGSGTQFTLTISDVVCDDAATYYCAGYKSSSTDGIAFGGGTEVVVK

SEQ ID NO: 10 - protein, 238 aa, synthetic construct
  REGION 1..238: note = Description of Artificial Sequence: Synthetic polypeptide
MDTRAPTQLLGLLLLWLPGATFAIVVTQTPSSKSVPVGGTVTINCQASESVYNSDWLAWYQQKPGQPPKQLIYAASTLASGVPSRFKGSGSGTQFTLTISDVVCDDAATYYCAGYKSSSTDGIAFGGGTEVVVKGDPVAPTVLIFPPAADQVATGTVTIVCVANKYFPDVTVTWEVDGTTQTTGIENSKTPQNSADCTYNLSSTLTLTSTQYNSHKEYTCKVTQGTTSVVQSFNRGDC

SEQ ID NO: 11 - protein, 13 aa, synthetic construct
  REGION 1..13: note = Description of Artificial Sequence: Synthetic peptide
QASESVYNSDWLA

SEQ ID NO: 12 - protein, 7 aa, synthetic construct
  REGION 1..7: note = Description of Artificial Sequence: Synthetic peptide
AASTLAS

SEQ ID NO: 13 - protein, 12 aa, synthetic construct
  REGION 1..12: note = Description of Artificial Sequence: Synthetic peptide
AGYKSSSTDGIA

SEQ ID NO: 14 - DNA, 396 bp, synthetic construct; identical to SEQ ID NO: 2
  misc_feature 1..396: note = Description of Artificial Sequence: Synthetic polynucleotide
  source 1..396: mol_type = other DNA

SEQ ID NO: 15 - protein, 132 aa, synthetic construct; identical to SEQ ID NO: 3
  REGION 1..132: note = Description of Artificial Sequence: Synthetic polypeptide

SEQ ID NO: 16 - protein, 455 aa, synthetic construct; identical to SEQ ID NO: 4
  REGION 1..455: note = Description of Artificial Sequence: Synthetic polypeptide

SEQ ID NO: 17 - DNA, 402 bp, synthetic construct
  misc_feature 1..402: note = Description of Artificial Sequence: Synthetic polynucleotide
  source 1..402: mol_type = other DNA
atggacacgagggcccccactcagctgctggggctcctgctgctctggctcccaggtgccacacttgccatcgtggtgacccagactccatcttccaagtctgtccctgtgggaggcacagtcaccatcaattgccaggccagtgagagtgtttataatagcgactggttagcctggtatcagcagaaaccagggcagcctcccaagcaactgatctatgctgcatccactctggcatctggggtcccatcgcgcttcaaaggcagtggatctgggacacagttcactctcaccatcagcgatgtggtgtgtgacgatgctgccacttattattgtgcaggatataaaagtagtagtactgatgggattgctttcggcggagggaccgaggtggtggtcaaa

SEQ ID NO: 18 - protein, 134 aa, synthetic construct
  REGION 1..134: note = Description of Artificial Sequence: Synthetic polypeptide
MDTRAPTQLLGLLLLWLPGATLAIVVTQTPSSKSVPVGGTVTINCQASESVYNSDWLAWYQQKPGQPPKQLIYAASTLASGVPSRFKGSGSGTQFTLTISDVVCDDAATYYCAGYKSSSTDGIAFGGGTEVVVK

SEQ ID NO: 19 - protein, 238 aa, synthetic construct
  REGION 1..238: note = Description of Artificial Sequence: Synthetic polypeptide
MDTRAPTQLLGLLLLWLPGATLAIVVTQTPSSKSVPVGGTVTINCQASESVYNSDWLAWYQQKPGQPPKQLIYAASTLASGVPSRFKGSGSGTQFTLTISDVVCDDAATYYCAGYKSSSTDGIAFGGGTEVVVKGDPVAPTVLIFPPAADQVATGTVTIVCVANKYFPDVTVTWEVDGTTQTTGIENSKTPQNSADCTYNLSSTLTLTSTQYNSHKEYTCKVTQGTTSVVQSFNRGDC

SEQ ID NO: 20 - DNA, 414 bp, synthetic construct
  misc_feature 1..414: note = Description of Artificial Sequence: Synthetic polynucleotide
  source 1..414: mol_type = other DNA
atggagactgggctgcgctggcttctcctggtcgctgtgctcaaaggtgtccagtgtcaggagcagctggaggagtccgggggaggcctggtcaagcctggggcatccctgacactcacctgcaaagcctctggattcgacttcagtatcaactactacatgtgctgggtccgccaggctccagggaaggggttggagtggatcgcatgcatttatactggtgatgatgacactttctacgcgagctgggcgaaaggccggttcaccatctccaaaacctcgtcgaccacggtgactctacaactgaacagtctgacagccgcggacacggccacctatttctgtgtgagaggtctatatagtggtagtattaataacctgtggggcccaggcaccctggtcaccgtctcctca

SEQ ID NO: 21 - protein, 138 aa, synthetic construct
  REGION 1..138: note = Description of Artificial Sequence: Synthetic polypeptide
METGLRWLLLVAVLKGVQCQEQLEESGGGLVKPGASLTLTCKASGFDFSINYYMCWVRQAPGKGLEWIACIYTGDDDTFYASWAKGRFTISKTSSTTVTLQLNSLTAADTATYFCVRGLYSGSINNLWGPGTLVTVSS

SEQ ID NO: 22 - protein, 461 aa, synthetic construct
  REGION 1..461: note = Description of Artificial Sequence: Synthetic polypeptide
METGLRWLLLVAVLKGVQCQEQLEESGGGLVKPGASLTLTCKASGFDFSINYYMCWVRQAPGKGLEWIACIYTGDDDTFYASWAKGRFTISKTSSTTVTLQLNSLTAADTATYFCVRGLYSGSINNLWGPGTLVTVSSGQPKAPSVFPLAPCCGDTPSSTVTLGCLVKGYLPEPVTVTWNSGTLTNGVRTFPSVRQSSGLYSLSSVVSVTSSSQPVTCNVAHPATNTKVDKTVAPSTCSKPTCPPPELLGGPSVFIFPPKPKDTLMISRTPEVTCVVVDVSQDDPEVQFTWYINNEQVRTARPPLREQQFNSTIRVVSTLPIAHQDWLRGKEFKCKVHNKALPAPIEKTISKARGQPLEPKVYTMGPPREELSSRSVSLTCMINGFYPSDISVEWEKNGKAEDNYKTTPAVLDSDGSYFLYSKLSVPTSEWQRGDVFTCSVMHEALHNHYTQKSISRSPGK

SEQ ID NO: 23 - protein, 8 aa, synthetic construct
  REGION 1..8: note = Description of Artificial Sequence: Synthetic peptide
GFDFSINY

SEQ ID NO: 24 - protein, 5 aa, synthetic construct
  REGION 1..5: note = Description of Artificial Sequence: Synthetic peptide
YTGDD

SEQ ID NO: 25 - protein, 10 aa, synthetic construct
  REGION 1..10: note = Description of Artificial Sequence: Synthetic peptide
GLYSGSINNL

SEQ ID NO: 26 - DNA, 402 bp, synthetic construct
  misc_feature 1..402: note = Description of Artificial Sequence: Synthetic polynucleotide
  source 1..402: mol_type = other DNA
atggacacgagggcccccactcagctgctggggctcctgctgctctggctcccagatgccagatgtgcgcttgtgatgacccagactccatcccctgtgtctgcagctgtgggaggcacagtcaccatcagttgccaggccagtcagagtgtttataacaacgactacttatcctggtatcagcagaaaccagggcagcctcccaaactcctgatctattatgcatccactctggcatctggggtctcatcgcggttcaaaggcagtggatctgggacacagttcactctcaccatcagcgacgtgcagtgtgacgatgctgccgcttactattgtgcaggcgttaaaggttatagtaatgataataatggtttcggcggagggaccgaggtggtggtcaaa

SEQ ID NO: 27 - protein, 134 aa, synthetic construct
  REGION 1..134: note = Description of Artificial Sequence: Synthetic polypeptide
MDTRAPTQLLGLLLLWLPDARCALVMTQTPSPVSAAVGGTVTISCQASQSVYNNDYLSWYQQKPGQPPKLLIYYASTLASGVSSRFKGSGSGTQFTLTISDVQCDDAAAYYCAGVKGYSNDNNGFGGGTEVVVK

SEQ ID NO: 28 - protein, 238 aa, synthetic construct
  REGION 1..238: note = Description of Artificial Sequence: Synthetic polypeptide
MDTRAPTQLLGLLLLWLPDARCALVMTQTPSPVSAAVGGTVTISCQASQSVYNNDYLSWYQQKPGQPPKLLIYYASTLASGVSSRFKGSGSGTQFTLTISDVQCDDAAAYYCAGVKGYSNDNNGFGGGTEVVVKGDPVAPTVLIFPPAADQVATGTVTIVCVANKYFPDVTVTWEVDGTTQTTGIENSKTPQNSADCTYNLSSTLTLTSTQYNSHKEYTCKVTQGTTSVVQSFNRGDC

SEQ ID NO: 29 - protein, 13 aa, synthetic construct
  REGION 1..13: note = Description of Artificial Sequence: Synthetic peptide
QASQSVYNNDYLS

SEQ ID NO: 30 - protein, 7 aa, synthetic construct
  REGION 1..7: note = Description of Artificial Sequence: Synthetic peptide
YASTLAS

SEQ ID NO: 31 - protein, 12 aa, synthetic construct
  REGION 1..12: note = Description of Artificial Sequence: Synthetic peptide
AGVKGYSNDNNG

SEQ ID NO: 32 - DNA, 411 bp, synthetic construct
  misc_feature 1..411: note = Description of Artificial Sequence: Synthetic polynucleotide
  source 1..411: mol_type = other DNA
atggagactgggctgcgctggcttctcctggtcgctgtgctcaaaggtgtccaatgtcagtcgctggaggagtccgggggaggcctggtcaagcctggggcatccctgacactcacctgcaaagcctctggattcgacttcagtatcaactactacatgtgctgggtccgccaggctccagggaaggggttggagtggatcgcatgcatttatactggtgatgatgacactttctacgcgagctgggcgaaaggccggttcaccatctccaaaacctcgtcgaccacggtgactctacaactgaacagtctgacagccgcggacacggccacctatttctgtgtgagaggtctatatagtggtagtattaataacctgtggggcccaggcaccctggtcaccgtctcctca

SEQ ID NO: 33 - protein, 137 aa, synthetic construct
  REGION 1..137: note = Description of Artificial Sequence: Synthetic polypeptide
METGLRWLLLVAVLKGVQCQSLEESGGGLVKPGASLTLTCKASGFDFSINYYMCWVRQAPGKGLEWIACIYTGDDDTFYASWAKGRFTISKTSSTTVTLQLNSLTAADTATYFCVRGLYSGSINNLWGPGTLVTVSS

SEQ ID NO: 34 - protein, 460 aa, synthetic construct
  REGION 1..460: note = Description of Artificial Sequence: Synthetic polypeptide
METGLRWLLLVAVLKGVQCQSLEESGGGLVKPGASLTLTCKASGFDFSINYYMCWVRQAPGKGLEWIACIYTGDDDTFYASWAKGRFTISKTSSTTVTLQLNSLTAADTATYFCVRGLYSGSINNLWGPGTLVTVSSGQPKAPSVFPLAPCCGDTPSSTVTLGCLVKGYLPEPVTVTWNSGTLTNGVRTFPSVRQSSGLYSLSSVVSVTSSSQPVTCNVAHPATNTKVDKTVAPSTCSKPTCPPPELLGGPSVFIFPPKPKDTLMISRTPEVTCVVVDVSQDDPEVQFTWYINNEQVRTARPPLREQQFNSTIRVVSTLPIAHQDWLRGKEFKCKVHNKALPAPIEKTISKARGQPLEPKVYTMGPPREELSSRSVSLTCMINGFYPSDISVEWEKNGKAEDNYKTTPAVLDSDGSYFLYSKLSVPTSEWQRGDVFTCSVMHEALHNHYTQKSISRSPGK

SEQ ID NO: 35 - DNA, 402 bp, synthetic construct; identical to SEQ ID NO: 26
  misc_feature 1..402: note = Description of Artificial Sequence: Synthetic polynucleotide
  source 1..402: mol_type = other DNA

SEQ ID NO: 36 - protein, 134 aa, synthetic construct; identical to SEQ ID NO: 27
  REGION 1..134: note = Description of Artificial Sequence: Synthetic polypeptide

SEQ ID NO: 37 - protein, 238 aa, synthetic construct; identical to SEQ ID NO: 28
  REGION 1..238: note = Description of Artificial Sequence: Synthetic polypeptide

SEQ ID NO: 38 - DNA, 417 bp, synthetic construct
  misc_feature 1..417: note = Description of Artificial Sequence: Synthetic polynucleotide
  source 1..417: mol_type = other DNA
atggagactgggctgcgctggcttctcctggtcgctgtgctcaaaggggtccagtgtcagtcgttggaggagtccgggggagacctggtcaagcctggggcatccctgacactcacctgcacagcctctggattctccttcacgagcaactactacatgtgctgggtccgccaggctccagggaaggggctggagtgggtcgcgtgcatttttcttggtagtagtggtaacactgtctacgcgaactgggcgaaaggccgattcaccatctccaaaacctcgtcgaccacggtgactctgcaaatgaccagtctgacagtcgcggacacggccacctatttctgtgcgagagactatgttaatggttatgactactttaacttgtggggcccaggcaccttggtcaccgtctcctca

SEQ ID NO: 39 - protein, 139 aa, synthetic construct
  REGION 1..139: note = Description of Artificial Sequence: Synthetic polypeptide
METGLRWLLLVAVLKGVQCQSLEESGGDLVKPGASLTLTCTASGFSFTSNYYMCWVRQAPGKGLEWVACIFLGSSGNTVYANWAKGRFTISKTSSTTVTLQMTSLTVADTATYFCARDYVNGYDYFNLWGPGTLVTVSS

SEQ ID NO: 40 - protein, 462 aa, synthetic construct
  REGION 1..462: note = Description of Artificial Sequence: Synthetic polypeptide
METGLRWLLLVAVLKGVQCQSLEESGGDLVKPGASLTLTCTASGFSFTSNYYMCWVRQAPGKGLEWVACIFLGSSGNTVYANWAKGRFTISKTSSTTVTLQMTSLTVADTATYFCARDYVNGYDYFNLWGPGTLVTVSSGQPKAPSVFPLAPCCGDTPSSTVTLGCLVKGYLPEPVTVTWNSGTLTNGVRTFPSVRQSSGLYSLSSVVSVTSSSQPVTCNVAHPATNTKVDKTVAPSTCSKPTCPPPELLGGPSVFIFPPKPKDTLMISRTPEVTCVVVDVSQDDPEVQFTWYINNEQVRTARPPLREQQFNSTIRVVSTLPIAHQDWLRGKEFKCKVHNKALPAPIEKTISKARGQPLEPKVYTMGPPREELSSRSVSLTCMINGFYPSDISVEWEKNGKAEDNYKTTPAVLDSDGSYFLYSKLSVPTSEWQRGDVFTCSVMHEALHNHYTQKSISRSPGK

SEQ ID NO: 41 - protein, 8 aa, synthetic construct
  REGION 1..8: note = Description of Artificial Sequence: Synthetic peptide
GFSFTSNY

SEQ ID NO: 42 - protein, 6 aa, synthetic construct
  REGION 1..6: note = Description of Artificial Sequence: Synthetic peptide
FLGSSG

SEQ ID NO: 43 - protein, 11 aa, synthetic construct
  REGION 1..11: note = Description of Artificial Sequence: Synthetic peptide
DYVNGYDYFNL

SEQ ID NO: 44 - DNA, 402 bp, synthetic construct
  misc_feature 1..402: note = Description of Artificial Sequence: Synthetic polynucleotide
  source 1..402: mol_type = other DNA
atggacacgagggcccccactcagctgctggggctcctgctgctctggctcccaggtgccacatttgcccaagtgctgacccagactgcatcccccgtgtctgcggctgttggaggcacagtcaccatcaattgccagtccagtcagagtgtttataataagaacttagcctggtatcagcagaaaccagggcagcctcccaaaggcctgatctattctacatcgactctagattctggggtcccatcgcggttcagcggcagtggatctgggacacagttcactctcaccatcagcgacgtgcagtgtgacgatgctgccacttactactgtctaggcagttatgattgtagtagtgctgattgtaatgctttcggcggagggaccgaggtggtggtcaaa

SEQ ID NO: 45 - protein, 134 aa, synthetic construct
  REGION 1..134: note = Description of Artificial Sequence: Synthetic polypeptide
MDTRAPTQLLGLLLLWLPGATFAQVLTQTASPVSAAVGGTVTINCQSSQSVYNKNLAWYQQKPGQPPKGLIYSTSTLDSGVPSRFSGSGSGTQFTLTISDVQCDDAATYYCLGSYDCSSADCNAFGGGTEVVVK

SEQ ID NO: 46 - protein, 238 aa, synthetic construct
  REGION 1..238: note = Description of Artificial Sequence: Synthetic polypeptide
MDTRAPTQLLGLLLLWLPGATFAQVLTQTASPVSAAVGGTVTINCQSSQSVYNKNLAWYQQKPGQPPKGLIYSTSTLDSGVPSRFSGSGSGTQFTLTISDVQCDDAATYYCLGSYDCSSADCNAFGGGTEVVVKGDPVAPTVLIFPPAADQVATGTVTIVCVANKYFPDVTVTWEVDGTTQTTGIENSKTPQNSADCTYNLSSTLTLTSTQYNSHKEYTCKVTQGTTSVVQSFNRGDC

SEQ ID NO: 47 - protein, 12 aa, synthetic construct
  REGION 1..12: note = Description of Artificial Sequence: Synthetic peptide
QSSQSVYNKNLA

SEQ ID NO: 48 - protein, 7 aa, synthetic construct
  REGION 1..7: note = Description of Artificial Sequence: Synthetic peptide
STSTLDS

SEQ ID NO: 49 - protein, 13 aa, synthetic construct
  REGION 1..13: note = Description of Artificial Sequence: Synthetic peptide
LGSYDCSSADCNA

SEQ ID NO: 50 - DNA, 399 bp, synthetic construct
  misc_feature 1..399: note = Description of Artificial Sequence: Synthetic polynucleotide
  source 1..399: mol_type = other DNA
atggagactgggctgcgctggcttctcctggtcgctgtgctcaaaggtgtccaatgtcagtcgctggaggagtccgggggaggcctggtcaagcctggggcatccctgacactcacctgcacagcctctggattctccttcagtgacagttggtacttgtgttgggtccgccaggctccagggaaggggctggagtggatcgcatgcatttatactggtgatggtgacacttattacgcgacctgggcgaaaggccgattcaccatctccaagacctcgtcgaccacagtgactctacaaatgaccagtctgacagccgcggacacggccacctatttctgtgcgaggggtgcccaattttacttgtggggccaaggcaccctggtcaccgtctcctca

SEQ ID NO: 51 - protein, 133 aa, synthetic construct
  REGION 1..133: note = Description of Artificial Sequence: Synthetic polypeptide
METGLRWLLLVAVLKGVQCQSLEESGGGLVKPGASLTLTCTASGFSFSDSWYLCWVRQAPGKGLEWIACIYTGDGDTYYATWAKGRFTISKTSSTTVTLQMTSLTAADTATYFCARGAQFYLWGQGTLVTVSS

SEQ ID NO: 52 - protein, 456 aa, synthetic construct
  REGION 1..456: note = Description of Artificial Sequence: Synthetic polypeptide
METGLRWLLLVAVLKGVQCQSLEESGGGLVKPGASLTLTCTASGFSFSDSWYLCWVRQAPGKGLEWIACIYTGDGDTYYATWAKGRFTISKTSSTTVTLQMTSLTAADTATYFCARGAQFYLWGQGTLVTVSSGQPKAPSVFPLAPCCGDTPSSTVTLGCLVKGYLPEPVTVTWNSGTLTNGVRTFPSVRQSSGLYSLSSVVSVTSSSQPVTCNVAHPATNTKVDKTVAPSTCSKPTCPPPELLGGPSVFIFPPKPKDTLMISRTPEVTCVVVDVSQDDPEVQFTWYINNEQVRTARPPLREQQFNSTIRVVSTLPIAHQDWLRGKEFKCKVHNKALPAPIEKTISKARGQPLEPKVYTMGPPREELSSRSVSLTCMINGFYPSDISVEWEKNGKAEDNYKTTPAVLDSDGSYFLYSKLSVPTSEWQRGDVFTCSVMHEALHNHYTQKSISRSPGK

SEQ ID NO: 53 - protein, 8 aa, synthetic construct
  REGION 1..8: note = Description of Artificial Sequence: Synthetic peptide
GFSFSDSW

SEQ ID NO: 54 - protein, 5 aa, synthetic construct
  REGION 1..5: note = Description of Artificial Sequence: Synthetic peptide
YTGDG

SEQ ID NO: 55 - protein, 6 aa, synthetic construct
  REGION 1..6: note = Description of Artificial Sequence: Synthetic peptide
GAQFYL

SEQ ID NO: 56 - DNA, 405 bp, synthetic construct
  misc_feature 1..405: note = Description of Artificial Sequence: Synthetic polynucleotide
  source 1..405: mol_type = other DNA
atggacacgagggcccccactcagctgctggggctcctgctgctctggctcccaggtgccacatttgcccaggtgctgacccagactccatcctccgtgtctgcagctgtgggaggcacagtcaccatcaattgccagtccagtcagagtgtttatgccaacacctacttatcctggtatcagcagaaaccagggcagcctcccaagcaactgatctattctgcatccagtctggcatctggggtcccaccgcggttcaaaggcagtggatctgggacacagttcgctctcaccatcagcgacgtgcagtgtgacgatgctgccacttactactgtctaggcagatatagttgtggtcttgctgattgtgctgctttcggcggagggaccgaggtggtggtcaaa

SEQ ID NO: 57 - protein, 135 aa, synthetic construct
  REGION 1..135: note = Description of Artificial Sequence: Synthetic polypeptide
MDTRAPTQLLGLLLLWLPGATFAQVLTQTPSSVSAAVGGTVTINCQSSQSVYANTYLSWYQQKPGQPPKQLIYSASSLASGVPPRFKGSGSGTQFALTISDVQCDDAATYYCLGRYSCGLADCAAFGGGTEVVVK

SEQ ID NO: 58 - protein, 239 aa, synthetic construct
  REGION 1..239: note = Description of Artificial Sequence: Synthetic polypeptide
MDTRAPTQLLGLLLLWLPGATFAQVLTQTPSSVSAAVGGTVTINCQSSQSVYANTYLSWYQQKPGQPPKQLIYSASSLASGVPPRFKGSGSGTQFALTISDVQCDDAATYYCLGRYSCGLADCAAFGGGTEVVVKGDPVAPTVLIFPPAADQVATGTVTIVCVANKYFPDVTVTWEVDGTTQTTGIENSKTPQNSADCTYNLSSTLTLTSTQYNSHKEYTCKVTQGTTSVVQSFNRGDC

SEQ ID NO: 59 - protein, 13 aa, synthetic construct
  REGION 1..13: note = Description of Artificial Sequence: Synthetic peptide
QSSQSVYANTYLS

SEQ ID NO: 60 - protein, 7 aa, synthetic construct
  REGION 1..7: note = Description of Artificial Sequence: Synthetic peptide
SASSLAS

SEQ ID NO: 61 - protein, 13 aa, synthetic construct
  REGION 1..13: note = Description of Artificial Sequence: Synthetic peptide
LGRYSCGLADCAA

SEQ ID NO: 62 - protein, 5 aa, synthetic construct
  REGION 1..5: note = Description of Artificial Sequence: Synthetic peptide
NNGIC

SEQ ID NO: 63 - protein, 17 aa, synthetic construct
  REGION 1..17: note = Description of Artificial Sequence: Synthetic peptide
CLYVGSSDTTYYASWAK

SEQ ID NO: 64 - protein, 6 aa, synthetic construct
  REGION 1..6: note = Description of Artificial Sequence: Synthetic peptide
INYYMC

SEQ ID NO: 65 - protein, 16 aa, synthetic construct
  REGION 1..16: note = Description of Artificial Sequence: Synthetic peptide
CIYTGDDDTFYASWAK

SEQ ID NO: 66 - protein, 6 aa, synthetic construct
  REGION 1..6: note = Description of Artificial Sequence: Synthetic peptide
SNYYMC

SEQ ID NO: 67 - protein, 17 aa, synthetic construct
  REGION 1..17: note = Description of Artificial Sequence: Synthetic peptide
CIFLGSSGNTVYANWAK

SEQ ID NO: 68 - protein, 6 aa, synthetic construct
  REGION 1..6: note = Description of Artificial Sequence: Synthetic peptide
DSWYLC

SEQ ID NO: 69 - protein, 16 aa, synthetic construct
  REGION 1..16: note = Description of Artificial Sequence: Synthetic peptide
CIYTGDGDTYYATWAK

SEQ ID NO: 70 - protein, 10 aa, synthetic construct
  REGION 1..10: note = Description of Artificial Sequence: Synthetic peptide
GFSFSNNGIC

SEQ ID NO: 71 - protein, 11 aa, synthetic construct
  REGION 1..11: note = Description of Artificial Sequence: Synthetic peptide
GFDFSINYYMC

SEQ ID NO: 72 - protein, 11 aa, synthetic construct
  REGION 1..11: note = Description of Artificial Sequence: Synthetic peptide
GFSFTSNYYMC

SEQ ID NO: 73 - protein, 11 aa, synthetic construct
  REGION 1..11: note = Description of Artificial Sequence: Synthetic peptide
GFSFSDSWYLC

SEQ ID NO: 74 - protein, 11 aa, synthetic construct
  REGION 1..11: note = Synthetic polypeptide
RASQDISKYLN

SEQ ID NO: 75 - protein, 7 aa, synthetic construct
  REGION 1..7: note = Synthetic polypeptide
HTSRLHS

SEQ ID NO: 76 - protein, 9 aa, synthetic construct
  REGION 1..9: note = Synthetic polypeptide
QQGNTLPYT

SEQ ID NO: 77 - protein, 7 aa, synthetic construct
  REGION 1..7: note = Synthetic polypeptide
GVSLPDY

SEQ ID NO: 78 - protein, 5 aa, synthetic construct
  REGION 1..5: note = Synthetic polypeptide
WGSET

SEQ ID NO: 79 - protein, 12 aa, synthetic construct
  REGION 1..12: note = Synthetic polypeptide
HYYYGGSYAMDY

SEQ ID NO: 80 - protein, 5 aa, synthetic construct
  REGION 1..5: note = Synthetic polypeptide
DYGVS

SEQ ID NO: 81 - protein, 16 aa, synthetic construct
  REGION 1..16: note = Synthetic polypeptide
VIWGSETTYYNSALKS

SEQ ID NO: 82 - protein, 10 aa, synthetic construct
  REGION 1..10: note = Synthetic polypeptide
GVSLPDYGVS